European Patent Specification EP 3 344 650 B1, published March 4, 2026. Title: AAV-EPO FOR TREATING COMPANION ANIMALS. Applicant: The Trustees of the University of Pennsylvania. The sequence listing filed with the application follows.

SEQUENCE LISTING (9 sequences)

SEQ ID NO: 1 - DNA, 5791 bp, Artificial Sequence
  constructed sequence
  misc_feature (12)..(629): Epo
  polyA_signal (696)..(822): Rabbit\globin\poly\A
  repeat_region (911)..(1040): 3' ITR (complement)
  rep_origin (1217)..(1672): f1/ori (complement)
  misc_feature (1803)..(2660): AP(R)
  rep_origin (2834)..(3422): origin of replication
  repeat_region (3862)..(3991): 5' ITR
  repeat_region (4059)..(4440): CMV\IE\promoter
  promoter (4443)..(4724): CB promoter
  TATA_signal (4697)..(4700)
  Intron (4819)..(5791): chicken\beta-actin\intron
aattcgccaccatgtgcgagcctgccccccctaagcctacacagtctgcctggcacagcttccccgagtgtcctgctctcctgctgctgctgagtttgctgctgctgcctctgggcctgcctgtgctgggagcacctcctagactgatctgcgacagccgggtgctggaacggtacatcctggaagcccgcgaggccgagaatgtgaccatgggatgtgcccagggctgcagcttcagcgagaacatcaccgtgcccgacaccaaagtgaacttctacacctggaagagaatggacgtgggccagcaggccctggaagtgtggcagggactggccctgctgtctgaggccatcctgagaggacaggctctgctggccaatgccagccagcctagcgagacacctcagctgcacgtggacaaggccgtgtcctccctgagaagcctgaccagcctgctgagagcactgggagcccagaaagaagccatgagcctgcctgaggaagccagccctgcccctctgagaaccttcaccgtggacaccctgtgcaagctgttccggatctacagcaacttcctgcggggcaagctgaccctgtacaccggcgaggcttgtcggagaggcgacagatgatgaggtacctctagagtcgacccgggcggcctcgaggacggggtgaactacgcctgaggatccgatctttttccctctgccaaaaattatggggacatcatgaagccccttgagcatctgacttctggctaataaaggaaatttattttcattgcaatagtgtgttggaattttttgtgtctctcactcggaagcaattcgttgatctgaatttcgaccacccataatacccattaccctggtagataagtagcatggcgggttaatcattaactacaaggaacccctagtgatggagttggccactccctctctgcgcgctcgctcgctcactgaggccgggcgaccaaaggtcgcccgacgcccgggctttgcccgggcggcctcagtgagcgagcgagcgcgcagccttaattaacctaattcactggccgtcgttttacaacgtcgtgactgggaaaaccctggcgttacccaacttaatcgccttgcagcacatccccctttcgccagctggcgtaatagcgaagaggcccgcaccgatcgcccttcccaacagttgcgcagcctgaatggcgaatgggacgcgccctgtagcggcgcattaagcgcggcgggtgtggtggttacgcgcagcgtgaccgctacacttgccagcgccctagcgcccgctcctttcgctttcttcccttcctttctcgccacgttcgccggctttccccgtcaagctctaaatcgggggctccctttagggttccgatttagtgctttacggcacctcgaccccaaaaaacttgattagggtgatggttcacgtagtgggccatcgccctgatagacggtttttcgccctttgacgttggagtccacgttctttaatagtggactcttgttccaaactggaacaacactcaaccctatctcggtctattcttttgatttataagggattttgccgatttcggcctattggttaaaaaatgagctgatttaacaaaaatttaacgcgaattttaacaaaatattaacgcttacaatttaggtggcacttttcggggaaatgtgcgcggaacccctatttgtttatttttctaaatacattcaaatatgtatccgctcatgagacaataaccctgataaatgcttcaataatattgaaaaaggaagagtatgagtattcaacatttccgtgtcgcccttattcccttttttgcggcattttgccttcctgtttttgctcacccagaaacgctggtgaaagtaaaagatgctgaagatcagttgggtgcacgagtgggttacatcgaactggatctcaacagcggtaagatccttgagagttttcgccccgaagaacgttttccaatgatgagcacttttaaagttctgctatgtggcgcggtattatcccgtattgacgccgggcaagagcaactcggtcgccgcatacactattctcagaatgacttggttgagtactcaccagtcacagaaaagcatcttacggatggcatgacagtaagagaattatgcagtgctgccataaccatgagtgataacactgcggccaacttacttctgacaacgatcggaggaccgaaggagctaaccgcttttttgcacaacatgggggatcatgtaactcgccttgatcgttgggaaccggagctgaatgaagccataccaaacgacgagcgtgacaccacgatgcctgtagcaatggcaacaacgttgcgcaaactattaactggcgaactacttactctagcttcccggcaacaattaatagactggatggaggcggataaagttgcaggaccacttctgcgctcggcccttccggctggctggtttattgctgataaatctggagccggtgagcgtgggtctcgcggtatcattgcagcactggggccagatggtaagccctcccgtatcgtagttatctacacgacggggagtcaggcaactatggatgaacgaaatagacagatcgctgagataggtgcctcactgattaagcattggtaactgtcagaccaagtttactcatatatactttagattgatttaaaacttcatttttaatttaaaaggatctaggtgaagatcctttttgataatctcatgaccaaaatcccttaacgtgagttttcgttccactgagcgtcagaccccgtagaaaagatcaaaggatcttcttgagatcctttttttctgcgcgtaatctgctgcttgcaaacaaaaaaaccaccgctaccagcggtggtttgtttgccggatcaagagctaccaactctttttccgaaggtaactggcttcagcagagcgcagataccaaatactgttcttctagtgtagccgtagttaggccaccacttcaagaactctgtagcaccgcctacatacctcgctctgctaatcctgttaccagtggctgctgccagtggcgataagtcgtgtcttaccgggttggactcaagacgatagttaccggataaggcgcagcggtcgggctgaacggggggttcgtgcacacagcccagcttggagcgaacgacctacaccgaactgagatacctacagcgtgagctatgagaaagcgccacgcttcccgaagggagaaaggcggacaggtatccggtaagcggcagggtcggaacaggagagcgcacgagggagcttccagggggaaacgcctggtatctttatagtcctgtcgggtttcgccacctctgacttgagcgtcgatttttgtgatgctcgtcaggggggcggagcctatggaaaaacgccagcaacgcggcctttttacggttcctggccttttgctggccttttgctcacatgttctttcctgcgttatcccctgattctgtggataaccgtattaccgcctttgagtgagctgataccgctcgccgcagccgaacgaccgagcgcagcgagtcagtgagcgaggaagcggaagagcgcccaatacgcaaaccgcctctccccgcgcgttggccgattcattaatgcagctggcacgacaggtttcccgactggaaagcgggcagtgagcgcaacgcaattaatgtgagttagctcactcattaggcaccccaggctttacactttatgcttccggctcgtatgttgtgtggaattgtgagcggataacaatttcacacaggaaacagctatgaccatgattacgccagatttaattaaggccttaattaggctgcgcgctcgctcgctcactgaggccgcccgggcaaagcccgggcgtcgggcgacctttggtcgcccggcctcagtgagcgagcgagcgcgcagagagggagtggccaactccatcactaggggttccttgtagttaatgattaacccgccatgctacttatctaccagggtaatggggatcctctagaactatagctagtcgacattgattattgactagttattaatagtaatcaattacggggtcattagttcatagcccatatatggagttccgcgttacataacttacggtaaatggcccgcctggctgaccgcccaacgacccccgcccattgacgtcaataatgacgtatgttcccatagtaacgccaatagggactttccattgacgtcaatgggtggactatttacggtaaactgcccacttggcagtacatcaagtgtatcatatgccaagtacgccccctattgacgtcaatgacggtaaatggcccgcctggcattatgcccagtacatgaccttatgggactttcctacttggcagtacatctacgtattagtcatcgctattaccatggtcgaggtgagccccacgttctgcttcactctccccatctcccccccctccccacccccaattttgtatttatttattttttaattattttgtgcagcgatgggggcggggggggggggggggcgcgcgccaggcggggcggggcggggcgaggggcggggcggggcgaggcggagaggtgcggcggcagccaatcagagcggcgcgctccgaaagtttccttttatggcgaggcggcggcggcggcggccctataaaaagcgaagcgcgcggcgggcggggagtcgctgcgacgctgccttcgccccgtgccccgctccgccgccgcctcgcgccgcccgccccggctctgactgaccgcgttactcccacaggtgagcgggcgggacggcccttctcctccgggctgtaattagcgcttggtttaatgacggcttgtttcttttctgtggctgcgtgaaagccttgaggggctccgggagggccctttgtgcggggggagcggctcggggggtgcgtgcgtgtgtgtgtgcgtggggagcgccgcgtgcggctccgcgctgcccggcggctgtgagcgctgcgggcgcggcgcggggctttgtgcgctccgcagtgtgcgcgaggggagcgcggccgggggcggtgccccgcggtgcggggggggctgcgaggggaacaaaggctgcgtgcggggtgtgtgcgtgggggggtgagcagggggtgtgggcgcgtcggtcgggctgcaaccccccctgcacccccctccccgagttgctgagcacggcccggcttcgggtgcggggctccgtacggggcgtggcgcggggctcgccgtgccgggcggggggtggcggcaggtgggggtgccgggcggggcggggccgcctcgggccggggagggctcgggggaggggcgcggcggcccccggagcgccggcggctgtcgaggcgcggcgagccgcagccattgccttttatggtaatcgtgcgagagggcgcagggacttcctttgtcccaaatctgtgcggagccgaaatctgggaggcgccgccgcaccccctctagcgggcgcggggcgaagcggtgcggcgccggcaggaaggaaatgggcggggagggccttcgtgcgtcgccgcgccgccgtccccttctccctctccagcctcggggctgtccgcggggggacggctgccttcgggggggacggggcagggcggggttcggcttctggcgtgtgaccggcggctctagagcctctgctaaccatgttcatgccttcttctttttcctacagctcctgggcaacgtgctggttattgtgctgtctcatcattttggcaaag

SEQ ID NO: 2 - DNA, 5749 bp, Artificial Sequence
  constructed sequence
  polyA_signal (56)..(182): Rabbit\globin\poly\A
  repeat_region (271)..(400): 3' ITR (complement)
  rep_origin (577)..(1032): F1 ori
  misc_feature (1163)..(2020): AP(R)
  rep_origin (2194)..(2782): Origin\of\replication
  repeat_region (3222)..(3351): 5' ITR
  repeat_region (3419)..(3800): CMV\IE\promoter
  promoter (3803)..(4084): CB promoter
  TATA_signal (4057)..(4060)
  Intron (4179)..(5151): chicken\beta-actin\intron
  misc_feature (5163)..(5738): Epo
ctctagagtcgacccgggcggcctcgaggacggggtgaactacgcctgaggatccgatctttttccctctgccaaaaattatggggacatcatgaagccccttgagcatctgacttctggctaataaaggaaatttattttcattgcaatagtgtgttggaattttttgtgtctctcactcggaagcaattcgttgatctgaatttcgaccacccataatacccattaccctggtagataagtagcatggcgggttaatcattaactacaaggaacccctagtgatggagttggccactccctctctgcgcgctcgctcgctcactgaggccgggcgaccaaaggtcgcccgacgcccgggctttgcccgggcggcctcagtgagcgagcgagcgcgcagccttaattaacctaattcactggccgtcgttttacaacgtcgtgactgggaaaaccctggcgttacccaacttaatcgccttgcagcacatccccctttcgccagctggcgtaatagcgaagaggcccgcaccgatcgcccttcccaacagttgcgcagcctgaatggcgaatgggacgcgccctgtagcggcgcattaagcgcggcgggtgtggtggttacgcgcagcgtgaccgctacacttgccagcgccctagcgcccgctcctttcgctttcttcccttcctttctcgccacgttcgccggctttccccgtcaagctctaaatcgggggctccctttagggttccgatttagtgctttacggcacctcgaccccaaaaaacttgattagggtgatggttcacgtagtgggccatcgccctgatagacggtttttcgccctttgacgttggagtccacgttctttaatagtggactcttgttccaaactggaacaacactcaaccctatctcggtctattcttttgatttataagggattttgccgatttcggcctattggttaaaaaatgagctgatttaacaaaaatttaacgcgaattttaacaaaatattaacgcttacaatttaggtggcacttttcggggaaatgtgcgcggaacccctatttgtttatttttctaaatacattcaaatatgtatccgctcatgagacaataaccctgataaatgcttcaataatattgaaaaaggaagagtatgagtattcaacatttccgtgtcgcccttattcccttttttgcggcattttgccttcctgtttttgctcacccagaaacgctggtgaaagtaaaagatgctgaagatcagttgggtgcacgagtgggttacatcgaactggatctcaacagcggtaagatccttgagagttttcgccccgaagaacgttttccaatgatgagcacttttaaagttctgctatgtggcgcggtattatcccgtattgacgccgggcaagagcaactcggtcgccgcatacactattctcagaatgacttggttgagtactcaccagtcacagaaaagcatcttacggatggcatgacagtaagagaattatgcagtgctgccataaccatgagtgataacactgcggccaacttacttctgacaacgatcggaggaccgaaggagctaaccgcttttttgcacaacatgggggatcatgtaactcgccttgatcgttgggaaccggagctgaatgaagccataccaaacgacgagcgtgacaccacgatgcctgtagcaatggcaacaacgttgcgcaaactattaactggcgaactacttactctagcttcccggcaacaattaatagactggatggaggcggataaagttgcaggaccacttctgcgctcggcccttccggctggctggtttattgctgataaatctggagccggtgagcgtgggtctcgcggtatcattgcagcactggggccagatggtaagccctcccgtatcgtagttatctacacgacggggagtcaggcaactatggatgaacgaaatagacagatcgctgagataggtgcctcactgattaagcattggtaactgtcagaccaagtttactcatatatactttagattgatttaaaacttcatttttaatttaaaaggatctaggtgaagatcctttttgataatctcatgaccaaaatcccttaacgtgagttttcgttccactgagcgtcagaccccgtagaaaagatcaaaggatcttcttgagatcctttttttctgcgcgtaatctgctgcttgcaaacaaaaaaaccaccgctaccagcggtggtttgtttgccggatcaagagctaccaactctttttccgaaggtaactggcttcagcagagcgcagataccaaatactgttcttctagtgtagccgtagttaggccaccacttcaagaactctgtagcaccgcctacatacctcgctctgctaatcctgttaccagtggctgctgccagtggcgataagtcgtgtcttaccgggttggactcaagacgatagttaccggataaggcgcagcggtcgggctgaacggggggttcgtgcacacagcccagcttggagcgaacgacctacaccgaactgagatacctacagcgtgagctatgagaaagcgccacgcttcccgaagggagaaaggcggacaggtatccggtaagcggcagggtcggaacaggagagcgcacgagggagcttccagggggaaacgcctggtatctttatagtcctgtcgggtttcgccacctctgacttgagcgtcgatttttgtgatgctcgtcaggggggcggagcctatggaaaaacgccagcaacgcggcctttttacggttcctggccttttgctggccttttgctcacatgttctttcctgcgttatcccctgattctgtggataaccgtattaccgcctttgagtgagctgataccgctcgccgcagccgaacgaccgagcgcagcgagtcagtgagcgaggaagcggaagagcgcccaatacgcaaaccgcctctccccgcgcgttggccgattcattaatgcagctggcacgacaggtttcccgactggaaagcgggcagtgagcgcaacgcaattaatgtgagttagctcactcattaggcaccccaggctttacactttatgcttccggctcgtatgttgtgtggaattgtgagcggataacaatttcacacaggaaacagctatgaccatgattacgccagatttaattaaggccttaattaggctgcgcgctcgctcgctcactgaggccgcccgggcaaagcccgggcgtcgggcgacctttggtcgcccggcctcagtgagcgagcgagcgcgcagagagggagtggccaactccatcactaggggttccttgtagttaatgattaacccgccatgctacttatctaccagggtaatggggatcctctagaactatagctagtcgacattgattattgactagttattaatagtaatcaattacggggtcattagttcatagcccatatatggagttccgcgttacataacttacggtaaatggcccgcctggctgaccgcccaacgacccccgcccattgacgtcaataatgacgtatgttcccatagtaacgccaatagggactttccattgacgtcaatgggtggactatttacggtaaactgcccacttggcagtacatcaagtgtatcatatgccaagtacgccccctattgacgtcaatgacggtaaatggcccgcctggcattatgcccagtacatgaccttatgggactttcctacttggcagtacatctacgtattagtcatcgctattaccatggtcgaggtgagccccacgttctgcttcactctccccatctcccccccctccccacccccaattttgtatttatttattttttaattattttgtgcagcgatgggggcggggggggggggggggcgcgcgccaggcggggcggggcggggcgaggggcggggcggggcgaggcggagaggtgcggcggcagccaatcagagcggcgcgctccgaaagtttccttttatggcgaggcggcggcggcggcggccctataaaaagcgaagcgcgcggcgggcggggagtcgctgcgacgctgccttcgccccgtgccccgctccgccgccgcctcgcgccgcccgccccggctctgactgaccgcgttactcccacaggtgagcgggcgggacggcccttctcctccgggctgtaattagcgcttggtttaatgacggcttgtttcttttctgtggctgcgtgaaagccttgaggggctccgggagggccctttgtgcggggggagcggctcggggggtgcgtgcgtgtgtgtgtgcgtggggagcgccgcgtgcggctccgcgctgcccggcggctgtgagcgctgcgggcgcggcgcggggctttgtgcgctccgcagtgtgcgcgaggggagcgcggccgggggcggtgccccgcggtgcggggggggctgcgaggggaacaaaggctgcgtgcggggtgtgtgcgtgggggggtgagcagggggtgtgggcgcgtcggtcgggctgcaaccccccctgcacccccctccccgagttgctgagcacggcccggcttcgggtgcggggctccgtacggggcgtggcgcggggctcgccgtgccgggcggggggtggcggcaggtgggggtgccgggcggggcggggccgcctcgggccggggagggctcgggggaggggcgcggcggcccccggagcgccggcggctgtcgaggcgcggcgagccgcagccattgccttttatggtaatcgtgcgagagggcgcagggacttcctttgtcccaaatctgtgcggagccgaaatctgggaggcgccgccgcaccccctctagcgggcgcggggcgaagcggtgcggcgccggcaggaaggaaatgggcggggagggccttcgtgcgtcgccgcgccgccgtccccttctccctctccagcctcggggctgtccgcggggggacggctgccttcgggggggacggggcagggcggggttcggcttctggcgtgtgaccggcggctctagagcctctgctaaccatgttcatgccttcttctttttcctacagctcctgggcaacgtgctggttattgtgctgtctcatcattttggcaaagaattcgccaccatgggcagctgcgagtgtcctgctctcctgctgctgctgagtttgctgctgctgcctctgggcctgcctgtgctgggagcacctcctagactgatctgcgacagccgggtgctggaacggtacatcctggaagcccgcgaggccgagaatgtgaccatgggatgtgccgagggctgcagcttcagcgagaacatcaccgtgcccgacaccaaagtgaacttctacacctggaagagaatggacgtgggccagcaggccgtggaagtgtggcagggactggccctgctgtctgaggccatcctgagaggacaggctctgctggccaacagcagccagcctagcgaaaccctgcagctgcacgtggacaaggccgtgtcctccctgagaagcctgaccagcctgctgagagcactgggagcccagaaagaggccacctctctgcctgaggccacatctgccgcccctctgagaaccttcaccgtggacaccctgtgcaagctgttccggatctacagcaacttcctgcggggcaagctgaccctgtacaccggcgaggcttgtcggagaggcgacagatgatgaggtac

SEQ ID NO: 3 - protein, 206 aa, Canis familiaris
MCEPAPPKPTQSAWHSFPECPALLLLLSLLLLPLGLPVLGAPPRLICDSRVLERYILEAREAENVTMGCAQGCSFSENITVPDTKVNFYTWKRMDVGQQALEVWQGLALLSEAILRGQALLANASQPSETPQLHVDKAVSSLRSLTSLLRALGAQKEAMSLPEEASPAPLRTFTVDTLCKLFRIYSNFLRGKLTLYTGEACRRGDR

SEQ ID NO: 4 - protein, 192 aa, Felis catus
MGSCECPALLLLLSLLLLPLGLPVLGAPPRLICDSRVLERYILEAREAENVTMGCAEGCSFSENITVPDTKVNFYTWKRMDVGQQAVEVWQGLALLSEAILRGQALLANSSQPSETLQLHVDKAVSSLRSLTSLLRALGAQKEATSLPEATSAAPLRTFTVDTLCKLFRIYSNFLRGKLTLYTGEACRRGDR

SEQ ID NO: 5 - DNA, 576 bp, Canis familiaris
atgggggcgtgcgaatgtcctgccctgttccttttgctgtctttgctgctgcttcctctgggcctcccagtcctgggcgccccccctcgcctcatttgtgacagccgggtcctggagagatacatcctggaggccagggaggccgaaaatgtcacgatgggctgtgctcaaggctgcagcttcagtgagaatatcaccgtcccagacaccaaggttaatttctatacctggaagaggatggatgttgggcagcaggccttggaagtctggcagggcctggcactgctctcagaagccatcctgcggggtcaggccctgttggccaacgcctcccagccatctgagactccgcagctgcatgtggacaaagccgtcagcagcctgcgcagcctcacctctctgcttcgggcgctgggagcccagaaggaggccatgtcccttccagaggaagcctctcctgctccactccgaacattcactgttgatactttgtgcaaacttttccgaatctactccaatttcctccgtggaaagctgacactgtacacaggggaggcctgcagaagaggagacagg

SEQ ID NO: 6 - DNA, 579 bp, Felis catus
atggggtcgtgcgaatgtcctgccctgctgcttctgctatctttgctgctgcttcccctgggcctcccagtcctgggcgccccccctcgcctcatctgtgacagccgagtcctggagaggtacattctgggggccagggaggccgaaaatgtcacgatgggctgtgctgaaggctgcagcttcagtgagaatatcactgtcccagacaccaaggtcaacttctatacctggaagaggatggacgtcgggcagcaggctgtggaagtctggcagggcctcgccctgctctcagaagccatcctgcggggccaggccctgctggccaactcctcccagccatctgagaccctgcagctgcatgtggataaagccgtcagcagcctgcgcagcctcacctccctgcttcgggcactgggagcccagaaggaagccacctcccttccagaggcaacctctgctgctccactccgaacattcactgtcgatactttgtgcaaacttttccgaatctactccaacttcctgcggggaaagctgacgctgtacacaggggaggcctgccgaagaggagacaggtga

SEQ ID NO: 7 - DNA, 618 bp, Artificial Sequence
  codon optimized sequence
atgtgcgagcctgccccccctaagcctacacagtctgcctggcacagcttccccgagtgtcctgctctcctgctgctgctgagtttgctgctgctgcctctgggcctgcctgtgctgggagcacctcctagactgatctgcgacagccgggtgctggaacggtacatcctggaagcccgcgaggccgagaatgtgaccatgggatgtgcccagggctgcagcttcagcgagaacatcaccgtgcccgacaccaaagtgaacttctacacctggaagagaatggacgtgggccagcaggccctggaagtgtggcagggactggccctgctgtctgaggccatcctgagaggacaggctctgctggccaatgccagccagcctagcgagacacctcagctgcacgtggacaaggccgtgtcctccctgagaagcctgaccagcctgctgagagcactgggagcccagaaagaagccatgagcctgcctgaggaagccagccctgcccctctgagaaccttcaccgtggacaccctgtgcaagctgttccggatctacagcaacttcctgcggggcaagctgaccctgtacaccggcgaggcttgtcggagaggcgacaga

SEQ ID NO: 8 - DNA, 576 bp, Artificial Sequence
  codon optimized sequence
atgggcagctgcgagtgtcctgctctcctgctgctgctgagtttgctgctgctgcctctgggcctgcctgtgctgggagcacctcctagactgatctgcgacagccgggtgctggaacggtacatcctggaagcccgcgaggccgagaatgtgaccatgggatgtgccgagggctgcagcttcagcgagaacatcaccgtgcccgacaccaaagtgaacttctacacctggaagagaatggacgtgggccagcaggccgtggaagtgtggcagggactggccctgctgtctgaggccatcctgagaggacaggctctgctggccaacagcagccagcctagcgaaaccctgcagctgcacgtggacaaggccgtgtcctccctgagaagcctgaccagcctgctgagagcactgggagcccagaaagaggccacctctctgcctgaggccacatctgccgcccctctgagaaccttcaccgtggacaccctgtgcaagctgttccggatctacagcaacttcctgcggggcaagctgaccctgtacaccggcgaggcttgtcggagaggcgacaga

SEQ ID NO: 9 - protein, 20 aa, Artificial Sequence
  IL-2 leader
MYRMQLLSCIALSLALVTNS